European Patent Application EP 4 353 820 A1, published April 17, 2024. Title: Superoxide dismutase 1 variant and method of producing glutathione or the derivative using thereof. Applicant: CJ CheilJedang Corporation. The sequence listing filed with the application follows.

SEQUENCE LISTING (30 sequences)

SEQ ID NO: 1 - protein, 154 aa, Saccharomyces cerevisiae
MVQAVAVLKGDAGVSGVVKFEQASESEPTTVSYEIAGNSPNAERGFHIHEFGDATNGCVSAGPHFNPFKKTHGAPTDEVRHVGDMGNVKTDENGVAKGSFKDSLIKLIGPTSVVGRSVVIHAGQDDLGKGDTEESLKTGNAGPRPACGVIGLTN

SEQ ID NO: 2 - DNA, 465 bp, Saccharomyces cerevisiae
atggttcaagcagtcgcagtgttaaagggtgatgccggtgtctctggtgttgtcaagttcgaacaggcttccgaatccgagccaaccactgtctcttacgagatcgctggtaacagtcctaacgcagaacgtgggttccacattcatgagtttggagatgccaccaatggttgtgtctctgctggtcctcacttcaatcctttcaagaagacacatggtgctccaactgacgaagtcagacatgtcggtgacatgggtaacgtaaagacggacgaaaatggtgtggccaagggctccttcaaggactctttgatcaagcttatcggtcctacctccgttgtaggcagaagcgtcgttatccacgccggccaagatgacttaggtaagggtgacactgaagaatctttgaagactggtaatgccggtccaagaccagcctgtggtgtcattggtctaaccaactaa

SEQ ID NO: 3 - DNA, 465 bp, Unknown
  Saccharomyces cerevisiae_CC02-2816_sod1
atggttcaagcagtcgcagtgttaaagggtgatgccggtgtctctggtgttgtcaagttcgaacaggcttccgaatccgagccaaccactgtctcttacgagatcgctggtaacagtcctaacgcagaacgtgggttccatattcatgagtttggagatgccaccaatggttgtgtctctgctggtcctcacttcaatcctttcaagaagacacacggtgctccaactgacgaagtcagacatgtcggtgacatgggtaacgtaaagacggacgaaaatggtgtggccaagggctccttcaaggactctttgatcaagcttatcggtcctacctccgttgtaggcagaagcgtcgttatccacgccggccaagatgacttaggtaagggtgacactgaagaatctttgaagactggtaatgccggtccaagaccagcctgtggtgtcattggtctaaccaactaa

SEQ ID NO: 4 - DNA, 35 bp, Artificial Sequence
  F_BamHI_SOD1
ggtaggatccatggttcaagcagtcgcagtgttaa

SEQ ID NO: 5 - DNA, 25 bp, Artificial Sequence
  F_SOD1_G37R
ttacgagatcgctcgcaacagtcct

SEQ ID NO: 6 - DNA, 25 bp, Artificial Sequence
  R_SOD1_G37R
aggactgttgcgagcgatctcgtaa

SEQ ID NO: 7 - DNA, 35 bp, Artificial Sequence
  R_XhoI_SOD1
atgactcgagttagttggttagaccaatgacacca

SEQ ID NO: 8 - DNA, 34 bp, Artificial Sequence
  F_SpeI_SOD1_DW
tagaactagttgttaatgataatatacttgaata

SEQ ID NO: 9 - DNA, 35 bp, Artificial Sequence
  R_NcoI_SOD1_DW
gctgccatggacactactagctcctgaagaccaag

SEQ ID NO: 10 - DNA, 27 bp, Artificial Sequence
  R_AL killer
gagcaatgaacccaataacgaaatctt

SEQ ID NO: 11 - DNA, 24 bp, Artificial Sequence
  F_BR killer
cttgacgttcgttcgactgatgag

SEQ ID NO: 12 - protein, 154 aa, Artificial Sequence
  SOD1 G37A
MVQAVAVLKGDAGVSGVVKFEQASESEPTTVSYEIAANSPNAERGFHIHEFGDATNGCVSAGPHFNPFKKTHGAPTDEVRHVGDMGNVKTDENGVAKGSFKDSLIKLIGPTSVVGRSVVIHAGQDDLGKGDTEESLKTGNAGPRPACGVIGLTN

SEQ ID NO: 13 - protein, 154 aa, Artificial Sequence
  SOD1 G37C
MVQAVAVLKGDAGVSGVVKFEQASESEPTTVSYEIACNSPNAERGFHIHEFGDATNGCVSAGPHFNPFKKTHGAPTDEVRHVGDMGNVKTDENGVAKGSFKDSLIKLIGPTSVVGRSVVIHAGQDDLGKGDTEESLKTGNAGPRPACGVIGLTN

SEQ ID NO: 14 - protein, 154 aa, Artificial Sequence
  SOD1 G37D
MVQAVAVLKGDAGVSGVVKFEQASESEPTTVSYEIADNSPNAERGFHIHEFGDATNGCVSAGPHFNPFKKTHGAPTDEVRHVGDMGNVKTDENGVAKGSFKDSLIKLIGPTSVVGRSVVIHAGQDDLGKGDTEESLKTGNAGPRPACGVIGLTN

SEQ ID NO: 15 - protein, 154 aa, Artificial Sequence
  SOD1 G37E
MVQAVAVLKGDAGVSGVVKFEQASESEPTTVSYEIAENSPNAERGFHIHEFGDATNGCVSAGPHFNPFKKTHGAPTDEVRHVGDMGNVKTDENGVAKGSFKDSLIKLIGPTSVVGRSVVIHAGQDDLGKGDTEESLKTGNAGPRPACGVIGLTN

SEQ ID NO: 16 - protein, 154 aa, Artificial Sequence
  SOD1 G37F
MVQAVAVLKGDAGVSGVVKFEQASESEPTTVSYEIAFNSPNAERGFHIHEFGDATNGCVSAGPHFNPFKKTHGAPTDEVRHVGDMGNVKTDENGVAKGSFKDSLIKLIGPTSVVGRSVVIHAGQDDLGKGDTEESLKTGNAGPRPACGVIGLTN

SEQ ID NO: 17 - protein, 154 aa, Artificial Sequence
  SOD1 G37H
MVQAVAVLKGDAGVSGVVKFEQASESEPTTVSYEIAHNSPNAERGFHIHEFGDATNGCVSAGPHFNPFKKTHGAPTDEVRHVGDMGNVKTDENGVAKGSFKDSLIKLIGPTSVVGRSVVIHAGQDDLGKGDTEESLKTGNAGPRPACGVIGLTN

SEQ ID NO: 18 - protein, 154 aa, Artificial Sequence
  SOD1 G37I
MVQAVAVLKGDAGVSGVVKFEQASESEPTTVSYEIAINSPNAERGFHIHEFGDATNGCVSAGPHFNPFKKTHGAPTDEVRHVGDMGNVKTDENGVAKGSFKDSLIKLIGPTSVVGRSVVIHAGQDDLGKGDTEESLKTGNAGPRPACGVIGLTN

SEQ ID NO: 19 - protein, 154 aa, Artificial Sequence
  SOD1 G37K
MVQAVAVLKGDAGVSGVVKFEQASESEPTTVSYEIAKNSPNAERGFHIHEFGDATNGCVSAGPHFNPFKKTHGAPTDEVRHVGDMGNVKTDENGVAKGSFKDSLIKLIGPTSVVGRSVVIHAGQDDLGKGDTEESLKTGNAGPRPACGVIGLTN

SEQ ID NO: 20 - protein, 154 aa, Artificial Sequence
  SOD1 G37L
MVQAVAVLKGDAGVSGVVKFEQASESEPTTVSYEIALNSPNAERGFHIHEFGDATNGCVSAGPHFNPFKKTHGAPTDEVRHVGDMGNVKTDENGVAKGSFKDSLIKLIGPTSVVGRSVVIHAGQDDLGKGDTEESLKTGNAGPRPACGVIGLTN

SEQ ID NO: 21 - protein, 154 aa, Artificial Sequence
  SOD1 G37M
MVQAVAVLKGDAGVSGVVKFEQASESEPTTVSYEIAMNSPNAERGFHIHEFGDATNGCVSAGPHFNPFKKTHGAPTDEVRHVGDMGNVKTDENGVAKGSFKDSLIKLIGPTSVVGRSVVIHAGQDDLGKGDTEESLKTGNAGPRPACGVIGLTN

SEQ ID NO: 22 - protein, 154 aa, Artificial Sequence
  SOD1 G37N
MVQAVAVLKGDAGVSGVVKFEQASESEPTTVSYEIANNSPNAERGFHIHEFGDATNGCVSAGPHFNPFKKTHGAPTDEVRHVGDMGNVKTDENGVAKGSFKDSLIKLIGPTSVVGRSVVIHAGQDDLGKGDTEESLKTGNAGPRPACGVIGLTN

SEQ ID NO: 23 - protein, 154 aa, Artificial Sequence
  SOD1 G37P
MVQAVAVLKGDAGVSGVVKFEQASESEPTTVSYEIAPNSPNAERGFHIHEFGDATNGCVSAGPHFNPFKKTHGAPTDEVRHVGDMGNVKTDENGVAKGSFKDSLIKLIGPTSVVGRSVVIHAGQDDLGKGDTEESLKTGNAGPRPACGVIGLTN

SEQ ID NO: 24 - protein, 154 aa, Artificial Sequence
  SOD1 G37Q
MVQAVAVLKGDAGVSGVVKFEQASESEPTTVSYEIAQNSPNAERGFHIHEFGDATNGCVSAGPHFNPFKKTHGAPTDEVRHVGDMGNVKTDENGVAKGSFKDSLIKLIGPTSVVGRSVVIHAGQDDLGKGDTEESLKTGNAGPRPACGVIGLTN

SEQ ID NO: 25 - protein, 154 aa, Artificial Sequence
  SOD1 G37R
MVQAVAVLKGDAGVSGVVKFEQASESEPTTVSYEIARNSPNAERGFHIHEFGDATNGCVSAGPHFNPFKKTHGAPTDEVRHVGDMGNVKTDENGVAKGSFKDSLIKLIGPTSVVGRSVVIHAGQDDLGKGDTEESLKTGNAGPRPACGVIGLTN

SEQ ID NO: 26 - protein, 154 aa, Artificial Sequence
  SOD1 G37S
MVQAVAVLKGDAGVSGVVKFEQASESEPTTVSYEIASNSPNAERGFHIHEFGDATNGCVSAGPHFNPFKKTHGAPTDEVRHVGDMGNVKTDENGVAKGSFKDSLIKLIGPTSVVGRSVVIHAGQDDLGKGDTEESLKTGNAGPRPACGVIGLTN

SEQ ID NO: 27 - protein, 154 aa, Artificial Sequence
  SOD1 G37T
MVQAVAVLKGDAGVSGVVKFEQASESEPTTVSYEIATNSPNAERGFHIHEFGDATNGCVSAGPHFNPFKKTHGAPTDEVRHVGDMGNVKTDENGVAKGSFKDSLIKLIGPTSVVGRSVVIHAGQDDLGKGDTEESLKTGNAGPRPACGVIGLTN

SEQ ID NO: 28 - protein, 154 aa, Artificial Sequence
  SOD1 G37V
MVQAVAVLKGDAGVSGVVKFEQASESEPTTVSYEIAVNSPNAERGFHIHEFGDATNGCVSAGPHFNPFKKTHGAPTDEVRHVGDMGNVKTDENGVAKGSFKDSLIKLIGPTSVVGRSVVIHAGQDDLGKGDTEESLKTGNAGPRPACGVIGLTN

SEQ ID NO: 29 - protein, 154 aa, Artificial Sequence
  SOD1 G37W
MVQAVAVLKGDAGVSGVVKFEQASESEPTTVSYEIAWNSPNAERGFHIHEFGDATNGCVSAGPHFNPFKKTHGAPTDEVRHVGDMGNVKTDENGVAKGSFKDSLIKLIGPTSVVGRSVVIHAGQDDLGKGDTEESLKTGNAGPRPACGVIGLTN

SEQ ID NO: 30 - protein, 155 aa, Artificial Sequence
  SOD1 G37Y
MVQAVAVLKGDAGVSGVVKFEQASESEPTTVSYEIAAYNSPNAERGFHIHEFGDATNGCVSAGPHFNPFKKTHGAPTDEVRHVGDMGNVKTDENGVAKGSFKDSLIKLIGPTSVVGRSVVIHAGQDDLGKGDTEESLKTGNAGPRPACGVIGLTN